European Patent Specification EP 3 887 375 B1, published November 20, 2024. Title: 3-(PHENYLSULFONYL)-[1,2,3]TRIAZOLO[1,5A]QUINAZOLIN-5(4H)-ONE DERIVATIVES. Applicant: Bioversys AG. The sequence listing filed with the application follows.

SEQUENCE LISTING (6 sequences)

SEQ ID NO: 1 - DNA, 25 bp, artificial sequence
  primer psma-fw
tatcaaaagcttaatcgaacaattc

SEQ ID NO: 2 - DNA, 25 bp, artificial sequence
  primer psma-rev
ccccttcaaataagatgttcatatc

SEQ ID NO: 3 - DNA, 20 bp, artificial sequence
  primer RNAIII-fw
ttcactgtgtcgataatcca

SEQ ID NO: 4 - DNA, 20 bp, artificial sequence
  primer RNAIII-rev
tgatttcaatggcacaagat

SEQ ID NO: 5 - DNA, 22 bp, artificial sequence
  primer rpoD-fw
gaggatcaggaagcacaaagtc

SEQ ID NO: 6 - DNA, 20 bp, artificial sequence
  primer rpoD-rev
gccgtcatcaagaccaaatc